European Patent Specification EP 4 045 493 B1, published August 13, 2025. Title: COMPOUNDS FOR TARGETED DEGRADATION OF CARRIER PROTEINS AND USES THEREOF. Applicant: CeMM - Forschungszentrum für Molekulare Medizin GmbH. The sequence listing filed with the application follows.

SEQUENCE LISTING (13 sequences)

SEQ ID NO: 1 - DNA, 2445 bp, Artificial Sequence
  SLC9A1, also denoted as P19634
atggtgctgcgctctggaatctgcggactgagcccacaccggatcttcccctccctgctggtggtggtggccctggtgggactgctgcctgtgctgagatctcacggactgcagctgagcccaaccgcatccacaatcaggagctccgagccacctagggagcggagcatcggcgacgtgaccacagcaccaccagaggtgacacctgagtccaggccagtgaaccactctgtgaccgatcacggcatgaagcctcggaaggccttcccagtgctgggcatcgactacacccacgtgagaacaccctttgagatcagcctgtggatcctgctggcctgcctgatgaagatcggcttccacgtgatccccacaatctctagcatcgtgcctgagtcctgtctgctgatcgtggtgggactgctggtgggaggactgatcaagggagtgggagagacccctccattcctgcagtctgacgtgttcttcctgttcctgctgccccctatcatcctggacgccggctacttcctgccactgaggcagtttaccgagaacctgggcacaatcctgatcttcgccgtggtgggcacactgtggaatgccttctttctgggcggcctgatgtatgccgtgtgcctggtgggaggagagcagatcaacaatatcggcctgctggataacctgctgtttggcagcatcatctccgccgtggacccagtggccgtgctggccgtgttcgaggagatccacatcaacgagctgctgcacatcctggtgtttggcgagtctctgctgaatgatgccgtgaccgtggtgctgtaccacctgttcgaggagtttgccaattatgagcacgtgggcatcgtggacatcttcctgggctttctgagcttctttgtggtggccctgggaggcgtgctggtgggagtggtgtacggcgtgatcgcagccttcacctctcggttcaccagccacatcagagtgatcgagcccctgttcgtgtttctgtacagctatatggcctatctgtccgccgagctgttccacctgtctggcatcatggcactgatcgcaagcggagtggtcatgcggccttacgtggaggccaatatctctcacaagagccacaccacaatcaagtattttctgaagatgtggtcctctgtgagcgagacactgatcttcatctttctgggcgtgagcaccgtggcaggatcccaccactggaactggaccttcgtgatctccacactgctgttttgcctgatcgcaagggtgctgggcgtgctgggactgacatggttcatcaataagtttcgcatcgtgaagctgacccccaaggatcagttcatcatcgcatacggaggactgagaggagcaatcgccttttccctgggctatctgctggataagaagcacttccctatgtgcgacctgtttctgaccgccatcatcacagtgatcttctttacagtgttcgtgcagggcatgaccatcaggccactggtggatctgctggccgtgaagaagaagcaggagaccaagcgcagcatcaacgaggagatccacacacagtttctggatcacctgctgaccggcatcgaggacatctgcggccactacggccaccaccactggaaggacaagctgaaccggttcaataagaagtatgtgaagaagtgtctgatcgccggcgagagatctaaggagcctcagctgatcgccttttaccacaagatggagatgaagcaggcaatcgagctggtggagagcggaggaatgggcaagatcccatccgccgtgtctaccgtgagcatgcagaatatccaccccaagtccctgccttctgagaggatcctgcccgccctgtccaaggataaggaggaggagatccgcaagatcctgcggaacaatctgcagaagacacggcagagactgaggtcttacaacaggcacaccctggtggccgacccatatgaggaggcctggaatcagatgctgctgcggagacagaaggcccgccagctggagcagaagatcaacaattacctgacagtgccagcccacaagctggattccccaaccatgtctagggcaaggatcggatccgacccactggcatatgagcctaaggaggatctgccagtgatcaccatcgacccagcaagcccacagtcccctgagtctgtggacctggtgaacgaggagctgaagggcaaggtgctgggactgagcagggatcctgcaaaggtggcagaggaggacgaggacgatgacggaggcatcatgatgagatccaaggagaccagctcccccggcacagatgacgtgttcaccccagccccctccgattctccttctagccagagaatccagaggtgcctgagcgaccctggaccacacccagagcctggagagggagagccattctttcccaagggccag

SEQ ID NO: 2 - DNA, 2436 bp, Artificial Sequence
  SLC9A2, also denoted as Q9UBYO
atggagcctctgggcaactggcgctccctgagggcaccactgccacctatgttattactgctgctgctgcaagtggcaggaccagtgggcgccctggccgagacactgctgaatgcacctagggcaatgggcaccagctcctctccaccaagcccagcatccgtggtggcaccaggaaccacactgttcgaggagagccggctgcccgtgtttacactggattaccctcacgtgcagatcccattcgagatcaccctgtggatcctgctggcctctctggccaagatcggctttcacctgtatcacaagctgccaacaatcgtgcccgagagctgcctgctgatcatggtgggcctgctgctgggcggcatcatcttcggcgtggatgagaagtcccctccagccatgaagaccgacgtgttctttctgtacctgctgccacctatcgtgctggacgcaggctatttcatgcccacccgccctttctttgagaacatcggcacaatcttttggtacgccgtggtgggcaccctgtggaattctatcggcatcggcgtgagcctgttcggcatttgtcaaatagaggcctttggcctgagcgatatcaccctgctgcagaacctgctgttcggctctctgatcagcgccgtggaccctgtggccgtgctggccgtgttcgagaacatccacgtgaatgagcagctgtacatcctggtgtttggcgagagcctgctgaacgatgccgtgaccgtggtgctgtataatctgttcaagtccttttgtcagatgaagaccatcgagacaatcgacgtgtttgccggcatcgccaacttctttgtggtgggaatcggaggcgtgctgatcggaatcttcctgggctttatcgccgccttcaccacacgctttacacacaatatcagagtgatcgagcccctgttcgtgtttctgtactcctatctgtcttacatcaccgccgagatgttccacctgtccggcatcatggccatcaccgcctgcgccatgacaatgaacaagtatgtggaggagaatgtgagccagaagtcctacaccacaatcaagtacttcatgaagatgctgagctccgtgtctgagacactgatcttcatctttatgggcgtgagcaccgtgggcaagaaccacgagtggaattgggccttcgtgtgctttacactggccttctgtctgatgtggagggccctgggcgtgttcgtgctgacccaggtcatcaaccgctttcggaccatcccactgacattcaaggaccagtttatcatcgcatacggaggactgaggggagcaatctgtttcgcactggtgtttctgctgccagcagccgtgttccctcggaagaagctgtttatcaccgccgccatcgtggtcatcttcttcaccgtgttcatcctgggcatcacaatcagacccctggtggagtttctggatgtgaagaggtctaataagaagcagcaggccgtgagcgaggagatctattgcagactgttcgatcacgtgaagaccggaatcgaggacgtgtgcggacactggggccacaacttttggagggacaagttcaagaagtttgacgataagtacctgagaaagctgctgatcagggagaatcagcctaagtctagcatcgtgtccctgtataagaagctggagatcaagcacgccatcgagatggccgagacaggcatgatcagcaccgtgccaacattcgcctccctgaacgattgtcgcgaggagaagatccggaaggtgacctcctctgagacagacgagatcagagagctgctgtccaggaacctgtaccagatcagacagaggaccctgagctataatcgccactccctgaccgccgatacatctgagcggcaggccaaggagatcctgatccggagaaggcactctctgagagagagcatcaggaaggacagctccctgaacagagagcacagggcctccacctctacaagcagatacctgagcctgcctaagaatacaaagctgccagagaagctgcagaagcgccggaccatcagcatcgccgatggcaactctagcgactccgatgcagacgcaggaaccacagtgctgaatctgcagccaagggccagaaggttcctgcccgagcagttttctaagaagagcccccagtcctataagatggagtggaagaatgaggtggatgtggactccggcagagacatgccctctaccccacccacacctcactccagggagaagggcacccagacatctggcctgctgcagcagcctctgctgtccaaggatcagtccggctctgagagagaggactctctgaccgagggcatccctccaaagccacctccaaggctggtgtggagggcatccgagccaggatctaggaaggcaaggttcggaagcgagaagccc

SEQ ID NO: 3 - DNA, 2502 bp, Artificial Sequence
  SLC9A3, also denoted as P48764
atgtggggcctgggcgccagaggcccagacaggggcctgctgctggccctggccctgggaggactggcaagggcaggaggcgtggaggtggagcccggcggcgcccacggcgagtctggcggctttcaggtggtgaccttcgagtgggcccacgtgcaggatccttatgtgatcgccctgtggatcctggtggcaagcctggccaagatcggcttccacctgtctcacaaggtgaccagcgtcgtgccagagtccgccctgctgatcgtgctgggactggtgctgggaggaatcgtgtgggccgccgaccacatcgccagctttaccctgacacccaccgtgttctttttctacctgctgccccctatcgtgctggatgccggctatttcatgcctaaccggctgtttttcggcaatctgggcacaatcctgctgtatgcagtggtgggaaccgtgtggaacgcagcaaccacaggactgagcctgtacggcgtgtttctgtccggactgatgggcgacctgcagatcggactgctggattttctgctgttcggaagcctgatggcagcagtggaccctgtggccgtgctggccgtgttcgaggaggtgcacgtgaacgaggtgctgtttatcatcgtgttcggcgagtccctgctgaacgatgccgtgacagtggtgctgtacaacgtgttcgagagttttgtcgcacttggtggggacaatgtgaccggcgtggattgcgtgaagggcatcgtgagcttcttcgtggtgagcctgggaggcacactggtgggcgtggtgtttgccttcctgctgtccctggtgacacgctttaccaagcacgtgcggatcatcgagcccggcttcgtgttcatcatctcctacctgtcttatctgacatctgagatgctgtctctgagcgccatcctggccatcaccttctgtggcatctgctgtcagaagtacgtgaaggccaacatcagcgagcagtccgccaccacagtgagatatacaatgaagatgctggccagctccgccgagaccatcatctttatgttcctgggcatcagcgccgtgaaccccttcatctggacatggaataccgcctttgtgctgctgacactggtgttcatctccgtgtacagggcaatcggagtggtgctgcagacctggctgctgaacagatataggatggtgcagctggagcccatcgaccaggtggtgctgtcctacggaggactgaggggagcagtggccttcgccctggtggtgctgctggacggcgataaggtgaaggagaagaatctgtttgtgagcaccacaatcatcgtggtgtttttcacagtgatcttccagggcctgaccatcaagccactggtgcagtggctgaaggtgaagagatccgagcacagggagccacggctgaacgagaagctgcacggcagggcctttgaccacatcctgtccgccatcgaggatatctctggccagatcggccacaattacctgagggacaagtggtcccactttgatcgcaagttcctgtctcgggtgctgatgcggagaagcgcccagaagtccagggaccggatcctgaacgtgttccacgagctgaatctgaaggatgccatcagctatgtggcagagggagagaggaggggatccctggcctttatcagatccccctctaccgacaacgtggtgaatgtggatttcacacctcgctctagcaccgtggaggccagcgtgtcctacctgctgcgggagaacgtgagcgccgtgtgcctggacatgcagtctctggagcagcggagaaggagcatcagggacgccgaggatatggtgacacaccacaccctgcagcagtacctgtataagcctagacaggagtacaagcacctgtattccaggcacgagctgacaccaaccgaggacgagaagcaggatagagagatctttcacaggacaatgagaaagaggctggagtctttcaagagcaccaagctgggcctgaaccagaataagaaggccgccaagctgtataagagggagagggcacagaagaggaggaactcctctatccctaatggcaagctgcctatggagtctccagcccagaacttcacaatcaaggagaaggacctggagctgagcgataccgaggagccacccaattacgacgaggagatgagcggcggcatcgagtttctggcctccgtgacaaaggacaccgcctctgatagcccagccggcatcgataatcccgtgttctctcctgacgaggccctggatcgcagcctgctggcaaggctgcctccatggctgtccccaggagagaccgtggtgccatctcagagagccaggacacagatcccatacagccccggcaccttttgtagactgatgcccttcaggctgagctccaagtccgtggactctttcctgcaggccgatggacctgaggagaggccacctgccgccctgccagagtccacccacatg

SEQ ID NO: 4 - DNA, 2394 bp, Artificial Sequence
  SLC9A4, also denoted as Q6AI14
atggccctgcagatgttcgtgacctactctccctggaactgcctgctgctgctggtggccctggagtgtagcgaggccagctccgatctgaacgagtctgccaatagcacagcccagtatgccagcaatgcatggttcgcagcagcatctagcgagccagaggagggcatctccgtgtttgagctggattacgactatgtgcagatcccctacgaggtgaccctgtggatcctgctggcctctctggccaagatcggcttccacctgtatcacaggctgcctggcctgatgccagagagctgcctgctgatcctggtgggcgccctggtgggaggcatcatctttggcaccgatcacaagtccccccctgtgatggactcctctatctacttcctgtatctgctgccaccaatcgtgctggagggaggatactttatgcccacacgccctttctttgagaacatcggctccatcctgtggtgggccgtgctgggcgccctgatcaatgcactgggcatcggcctgtctctgtatctgatctgtcaggtgaaggccttcggcctgggcgatgtgaacctgctgcagaatctgctgtttggctccctgatctctgccgtggaccctgtggccgtgctggccgtgttcgaggaggcacgggtgaacgagcagctgtacatgatgatctttggcgaggccctgctgaacgacggcatcaccgtggtgctgtataatatgctgatcgccttcaccaagatgcacaagtttgaggatatcgagacagtggacatcctggcaggatgcgcaaggttcatcgtggtgggactgggaggcgtgctgtttggcatcgtgttcggctttatctccgccttcatcacccgctttacacagaacatctctgccatcgagcccctgatcgtgttcatgtttagctacctgtcctatctggcagcagagaccctgtacctgtccggaatcctggcaatcaccgcatgtgcagtgacaatgaagaagtatgtggaggagaacgtgagccagacaagctacaccacaatcaagtatttcatgaagatgctgagctccgtgagcgagaccctgatcttcatctttatgggcgtgtccacagtgggcaagaaccacgagtggaattgggccttcatctgctttaccctggccttttgtcagatctggcgggccatcagcgtgttcgccctgttttacatcagcaaccagttcagaacattccctttttctatcaaggatcagtgcatcatcttttatagcggcgtgaggggagcaggatctttcagcctggcctttctgctgcctctgagcctgttcccacgcaagaagatgtttgtgaccgccacactggtggtcatctacttcaccgtgttcatccagggcatcacagtgggcccactggtgcggtatctggacgtgaagaagaccaacaagaaggagtccatcaatgaggagctgcacatcagactgatggatcacctgaaggcaggaatcgaggacgtgtgcggacactggagccactaccaggtgagggataagttcaagaagtttgaccacaggtatctgcgcaagatcctgatccgcaagaatctgcccaagtctagcatcgtgtccctgtacaagaagctggagatgaagcaggccatcgagatggtggagaccggcatcctgtcctctacagccttcagcatcccccaccaggcccagaggatccagggcatcaagcgcctgtctcctgaggatgtggagagcatcagagacatcctgacctctaacatgtaccaggtgcggcagagaacactgagctacaacaagtataatctgaagcctcagacctccgagaagcaggccaaggagatcctgatccggagacagaatacactgagggagtccatgcgcaagggacactctctgccatggggcaagcctgcaggaaccaagaacatccggtacctgtcctacccatatggcaatccccagtctgccggaagggataccagagcagcaggcttcagcgacgatgacagctccgacccaggctccccctctatcacattttccgcctgctctagaatcggctccctgcagaagcaggaggcccaggagatcatcccaatgaagtctctgcacaggggccgcaaggccttcagctttggctaccagcggaacacctcccaggaggagtatctgggaggcgtgaggagggtggccctgagacctaagccactgttccacgcagtggatgaggagggagagagcggaggagagtccgagggcaaggcaagcctggtggaggtgcggtccagatggacagcagatcacggacacggaagggaccaccacagaagccactcccccctgctgcagaagaag

SEQ ID NO: 5 - DNA, 2688 bp, Artificial Sequence
  SLCA5, also denoted as Q14940
atgctgagagccgccctgtctctgctggccctgccactggcaggagcagcagaggagcctacccagaagccagagagcccaggagagccacctccaggactggagctgttcagatggcagtggcacgaggtggaggcaccatacctggtggccctgtggatcctggtggcaagcctggccaagatcgtgtttcacctgtctaggaaggtgaccagcctggtgcctgagtcctgcctgctgatcctgctgggactggtgctgggaggaatcgtgctggccgtggccaagaaggccgagtatcagctggagccaggcacattctttctgttcctgctgccccctatcgtgctggactccggctactttatgccctctcgcctgttctttgataacctgggcgccatcctgacctacgcagtggttgggactttgtggaatgccttcaccacaggagccgccctgtggggactgcagcaggcaggcctggtggcccctagggtgcaggcaggactgctggacttcctgctgtttggcagcctgatctccgccgtggatccagtggccgtgctggccgtgtttgaggaggtgcacgtgaacgagaccctgttcatcatcgtgtttggcgagagcctgctgaatgacgccgtgacagtggtgctgtacaaggtgtgcaacagcttcgtggagatgggctccgccaatgtgcaggccaccgattatctgaagggcgtggcctctctgtttgtggtgagcctgggaggagcagcagtgggactggtgttcgcctttctgctggccctgaccacaagattcacaaagagagtgaggatcatcgagcctctgctggtgtttctgctggcctacgccgcctatctgaccgccgagatggcctctctgagcgccatcctggccgtgacaatgtgcggcctgggctgtaagaagtacgtggaggccaacatctctcacaagagcaggaccacagtgaagtataccatgaagacactggcctcctgtgccgagaccgtgatcttcatgctgctgggcatctccgccgtggacagctccaagtgggcatgggattctggcctggtgctgggcaccctgatcttcatcctgttctttcgcgccctgggagtggtgctgcagacatgggtgctgaatcagtttcggctggtgccactggacaagatcgatcaggtggtcatgagctacggaggactgaggggagcagtggccttcgccctggtcatcctgctggaccggaccaaggtgcccgccaaggattattttgtggccaccacaatcgtggtggtgttctttaccgtgatcgtgcagggcctgacaatcaagcccctggtgaagtggctgaaggtgaagcggtccgagcaccacaagcctaccctgaaccaggagctgcacgagcacacattcgaccacatcctggcagcagtggaggatgtggtgggacaccacggctaccactattggcgcgaccggtgggagcagtttgataagaagtacctgtcccagctgctgatgcggagatctgcctatagaatcagggaccagatctgggacgtgtactatcgcctgaatatccgggacgccatcagcttcgtggatcagggaggacacgtgctgtctagcaccggactgacactgccttccatgccatctagaaacagcgtggccgagacctccgtgacaaatctgctgagggagtccggatctggagcatgcctggacctgcaggtcatcgataccgtgcgctctggaagggacagggaggatgccgtgatgcaccacctgctgtgcggaggactgtacaagccaaggcgccggtataaggccagctgttccagacacttcatctctgaggacgcccaggagaggcaggataaggaggtgtttcagcagaacatgaagagaaggctggagtccttcaagtctaccaagcacaatatctgttttacaaagtccaagcctagaccaaggaagaccggccgccggaagaaggacggagtggcaaacgcagaggcaacaaatggcaagcacaggggactgggattccaggacaccgcagccgtgatcctgacagtggagagcgaggaggaggaggaggagtccgattcctctgagaccgagaaggaggacgatgagggcatcatctttgtggcaagggccacaagcgaggtgctgcaggagggcaaggtgtctggaagcctggaggtgtgcccatctcctaggatcatcccacccagcccaacctgtgccgagaaggagctgccatggaagagcggacagggcgacctggccgtgtacgtgagctccgagaccacaaagatcgtgcctgtggatatgcagacaggctggaaccagtccatctctagcctggagagcctggcctcccctccatgcaatcaggcccctatcctgacctgtctgccccctcacccaagaggcacagaggagccccaggtgcctctgcacctgccaagcgaccccaggtcctctttcgcctttccaccatccctggcaaaggcaggccgctcccggtctgagagctccgccgacctgcctcagcagcaggagctgcagccactgatgggccacaaggatcacacccacctgtctccaggcaccgccacaagccactggtgtatccagttcaacagaggctccaggctg

SEQ ID NO: 6 - DNA, 2007 bp, Artificial Sequence
  SLCA6, also denoted as Q92581
atggctcggagaggctggaggcgcgcccctctgcggagaggagtgggaagctcccctagggcaaggcgcctgatgagaccactgtggctgctgctggcagtgggcgtgttcgattgggcaggagcatctgacggaggaggaggagaggcccgggccatggatgaggagatcgtgagcgagaagcaggccgaggagtcccacagacaggactctgccaatctgctgatcttcatcctgctgctgacactgaccatcctgaccatctggctgtttaagcaccggagagccaggttcctgcacgagacaggcctggccatgatctacggactgctggtgggactggtgctgcgctatggcatccacgtgccatccgatgtgaacaatgtgaccctgtcttgcgaggtgcagtctagccccaccacactgctggtgacattcgaccctgaggtgttctttaatatcctgctgccccctatcatcttttacgccggctattccctgaagaggcgccacttctttcggaacctgggctctatcctggcctacgcctttctgggcaccgccatcagctgcttcgtgatcggctccatcatgtatggctgcgtgaccctgatgaaggtgaccggccagctggccggcgatttctactttaccgactgtctgctgttcggcgccatcgtgtccgccacagatccagtgaccgtgctggccatcttccacgagctgcaggtggacgtggagctgtatgccctgctgtttggcgagagcgtgctgaatgacgccgtggccatcgtgctgtcctctagcatcgtggcataccagccagcaggcgataactctcacacatttgacgtgaccgccatgttcaagagcatcggcatcttcctgggcatcttttctggcagcttcgccatgggagcagcaacaggagtggtgaccgccctggtgacaaagtttaccaagctgagggagttccagctgctggagacaggcctgttctttctgatgtcctggtctacctttctgctggcagaggcatggggcttcacaggagtggtggccgtgctgttttgcggcatcacacaggcccactacacctataacaatctgagcacagagtcccagcaccgcaccaagcagctgtttgagctgctgaacttcctggccgagaatttcatcttttcctatatgggcctgacactgttcacctttcagaaccacgtgtttaatcctaccttcgtggtgggcgcctttgtggccatcttcctgggcagggccgccaacatctacccactgagcctgctgctgaatctgggccggagatctaagatcggcagcaattttcagcacatgatgatgttcgcaggactgaggggagcaatggccttcgccctggccatcagggatacagccacctacgcccgccagatgatgttctccaccacactgctgatcgtgttctttaccgtgtgggtgtttggaggaggaaccacagcaatgctgagctgcctgcacatccgggtgggcgtggattccgaccaggagcacctgggagtgccagagaacgagaggaggaccacaaaggcagagtccgcctggctgtttagaatgtggtacaacttcgaccacaattatctgaagccactgctgacccactctggaccaccactgaccacaaccctgccagcatgctgtggacctatcgcaagatgtctgaccagccctcaggcctatgagaaccaggagcagctgaaggacgatgactccgatctgatcctgaatgatggcgacatctctctgacctacggcgacagcacagtgaacaccgagccagccacatcctctgccccacggagattcatgggcaacagctccgaggatgcactggacagggagctggcctttggcgatcacgagctggtcatcaggggaaccaggctggtgctgccaatggatgacagcgagcctccactgaacctgctggacaatacaagacacggccccgcc

SEQ ID NO: 7 - DNA, 1743 bp, Artificial Sequence
  SLCA8, also denoted as Q9Y2E8
atgggcgagaagatggccgaggaggagcggttcccaaacaccacacacgagggctttaatgtgacactgcacaccacactggtggtgaccacaaagctggtgctgccaacacccggcaagcctatcctgccagtgcagaccggagagcaggcacagcaggaggagcagagctccggcatgaccatcttctttagcctgctggtgctggccatctgcatcatcctggtgcacctgctgatcaggtacaggctgcacttcctgccagagtccgtggcagtggtgtctctgggcatcctgatgggcgccgtgatcaagatcatcgagttcaagaagcttgccaactggaaagaggaggagatgtttagacctaacatgttctttctgctgctgctgccccctatcatcttcgagagcggctactccctgcacaagggcaacttctttcagaatatcggctccatcacactgttcgccgtgtttggcaccgcaatctctgccttcgtggtgggaggaggcatctattttctgggccaggccgacgtgatctctaagctgaatatgacagatagcttcgcctttggctctctgatcagcgccgtggacccagtggcaaccatcgccatcttcaacgccctgcacgtggatcccgtgctgaatatgctggtgtttggcgagtccatcctgaacgacgccgtgtctatcgtgctgacaaataccgccgagggcctgacaaggaagaacatgtccgacgtgtctggctggcagaccttcctgcaggccctggattactttctgaagatgttctttggaagcgccgccctgggcacactgaccggactgatctccgccctggtgctgaagcacatcgatctgcgcaagacccctagcctggagttcggcatgatgatcatctttgcctacctgccatatggactggcagagggaatctctctgagcggaatcatggccatcctgttcagcggcatcgtgatgtcccactatacacaccacaacctgtccccagtgacccagatcctgatgcagcagacactgaggaccgtggcctttctgtgcgagacctgcgtgttcgcctttctgggcctgagcatcttctcctttccccacaagttcgagatcagctttgtgatctggtgtatcgtgctggtgctgttcggccgggccgtgaatatctttcccctgtcctacctgctgaacttctttagagaccacaagatcacccctaagatgatgttcatcatgtggttttctggactgaggggagcaatcccatatgcactgagcctgcacctggatctggagcctatggagaagagacagctgatcggcaccacaaccatcgtgatcgtgctgttcacaatcctgctgctgggcggctctaccatgcctctgatcagactgatggacatcgaggatgccaaggcccaccggagaaacaagaaggacgtgaatctgtccaagacagagaagatgggcaataccgtggagtctgagcacctgagcgagctgaccgaggaggagtacgaggcccactatatcaggcgccaggacctgaagggcttcgtgtggctggatgccaagtacctgaatcctttctttacacggagactgacccaggaggatctgcaccacggcaggatccagatgaagacactgaccaacaagtggtatgaggaggtgcgccagggaccatccggatctgaggacgatgagcaggagctgctg

SEQ ID NO: 8 - DNA, 1935 bp, Artificial Sequence
  SLCA9, also denoted as Q8IVB4
atggagaggcagtctcgcgtgatgagcgagaaggacgagtaccagtttcagcaccagggagcagtggagctgctggtgttcaactttctgctgatcctgaccatcctgacaatctggctgttcaagaatcaccggttcagatttctgcacgagaccggcggcgccatggtgtatggcctgatcatgggactgatcctgagatacgcaaccgcaccaacagacatcgagagcggaaccgtgtacgattgcgtgaagctgaccttcagcccttccacactgctggtgaacatcacagaccaggtgtacgagtataagtacaagcgcgagatctcccagcacaacatcaatccccaccagggcaacgccatcctggagaagatgacctttgatcctgagatcttctttaatgtgctgctgccccctatcatcttccacgccggctattccctgaagaagcggcacttctttcagaacctgggctctatcctgacctacgcctttctgggcacagccatcagctgcatcgtgatcggcctgatcatgtatggcttcgtgaaggccatgatccacgccggccagctgaagaatggcgacttccactttaccgattgtctgttctttggcagcctgatgtccgccaccgacccagtgacagtgctggccatctttcacgagctgcacgtggaccccgatctgtacaccctgctgttcggagagtccgtgctgaacgacgcagtggccatcgtgctgacatattctatcagcatctacagcccaaaggagaaccccaatgccttcgatgccgccgccttctttcagtccgtgggcaatttcctgggcatctttgccggctccttcgccatgggctctgcctatgccatcatcaccgccctgctgaccaagtttacaaagctgtgcgagttccccatgctggagacaggcctgttctttctgctgtcctggtctgcctttctgtccgccgaggcagcaggactgaccggaatcgtggccgtgctgttctgtggcgtgacccaggcccactatacatacaacaatctgagctccgattctaagatcaggaccaagcagctgttcgagtttatgaactttctggccgagaatgtgatcttctgctacatgggcctggccctgttcacatttcagaaccacatctttaatgccctgttcatcctgggcgcctttctggccatcttcgtggcccgggcctgtaacatctatcctctgagctttctgctgaatctgggcagaaagcagaagatcccatggaactttcagcacatgatgatgttctctggactgaggggagcaatcgccttcgccctggccatccgcaataccgagagccagcccaagcagatgatgtttaccacaaccctgctgctggtgttctttaccgtgtgggtgttcggaggaggaacaaccccaatgctgacatggctgcagatcagggtgggagtggacctggatgagaacctgaaggaggacccctctagccagcaccaggaggccaacaatctggataagaatatgacaaaggccgagtctgcccggctgtttagaatgtggtatagcttcgaccacaagtacctgaagcctatcctgacccactctggcccacccctgacaaccacactgcctgagtggtgtggcccaatcagccggctgctgacatccccacaggcctacggcgagcagctgaaggaggacgatgtggagtgcatcgtgaaccaggatgagctggccatcaattatcaggagcaggcctcctctccttgttcccctccagccagactgggcctggaccagaaggcctctccccagacccctggcaaggagaacatctatgagggcgatctgggactgggaggatacgagctgaagctggagcagacactgggccagagccagctgaat

SEQ ID NO: 9 - DNA, 1611 bp, Artificial Sequence
  SLCB2, also denoted as Q86UD5
atgggcgacgaggataagcggatcacctacgaggactccgagccatctaccggcatgaactatacaccctctatgcaccaggaggcccaggaggagaccgtgatgaagctgaagggcatcgatgccaatgagccaacagagggcagcatcctgctgaagagctccgagaagaagctgcaggagaccccaacagaggcaaaccacgtgcagcggctgagacagatgctggcatgcccacctcacggactgctggacagagtgatcaccaatgtgacaatcatcgtgctgctgtgggccgtggtgtggtccatcaccggatctgagtgcctgccaggaggaaacctgttcggcatcatcatcctgttttactgtgccatcatcggcggcaagctgctgggcctgatcaagctgcccacactgccacccctgccttccctgctgggaatgctgctggcaggcttcctgatcaggaatatccccgtgatcaacgacaatgtgcagatcaagcacaagtggtctagctccctgcggagcatcgccctgtccatcatcctggtgagagccggcctgggcctggattctaaggccctgaagaagctgaagggcgtgtgcgtgcgcctgtctatgggaccttgcatcgtggaggcatgtaccagcgccctgctggcacactacctgctgggactgccatggcagtggggcttcatcctgggctttgtgctgggagccgtgtctcctgcagtggtggtgccaagcatgctgctgctgcagggaggaggatatggagtggagaagggagtgcctacactgctgatggcagcaggctccttcgacgatatcctggccatcaccggctttaacacatgtctgggcatcgccttcagcaccggctccacagtgtttaatgtgctgaggggcgtgctggaggtggtcatcggagtggcaaccggatccgtgctgggcttctttatccagtacttcccctctagggaccaggataagctggtgtgcaagcgcacattcctggtgctgggactgagcgtgctggccgtgttttctagcgtgcacttcggatttcctggatccggaggactgtgcaccctggtcatggcctttctggccggcatgggctggacatccgagaaggccgaggtggagaagatcatcgccgtggcctgggatatcttccagcccctgctgtttggcctgatcggcgccgaggtgtctatcgcaagcctgaggcctgagaccgtgggactgtgcgtggcaacagtgggaatcgccgtgctgatccgcatcctgaccacattcctgatggtgtgcttcgccggctttaacctgaaggagaagatcttcatcagctttgcctggctgcccaaggccaccgtgcaggcagcaatcggatccgtggccctggacacagcacggtctcacggcgagaagcagctggaggactatggcatggatgtgctgaccgtggcctttctgagcatcctgatcacagcccctatcggatccctgctgatcggactgctgggaccaagactgctgcagaaggtggagcaccagaataaggatgaggaggtgcagggcgagaccagcgtgcaggtg

SEQ ID NO: 10 - DNA, 86 bp, Artificial Sequence
  SLC38A2_5-PITCH
cgcgttacatagcatcgtacgcgtacgtgtttggtagcttgaagaaggccgaaaccatggccaagcctttgtctcaagaagaatcc

SEQ ID NO: 11 - DNA, 95 bp, Artificial Sequence
  SLC38A2_3-PITCH
catcagcattctagagcatcgtacgcgtacgtgtttggggggaaatactgaatcgtcccatctctgctttcttcatagatccgccgccacccgac

SEQ ID NO: 12 - DNA, 25 bp, Artificial Sequence
  SLC38A2_gRNA_S
caccgaatactgaatcgtcccattt

SEQ ID NO: 13 - DNA, 25 bp, Artificial Sequence
  SLC38A2_gRNA_AS
aaacaaatgggacgattcagtattc